European Patent Specification EP 3 448 369 B1, published June 25, 2025. Title: Compounds and Compositions Useful for Treating Metabolic Syndrome, and Methods Using Same. Applicant: THE REGENTS OF THE UNIVERSITY OF COLORADO, A BODY CORPORATE McKinsey, Timothy Bagchi, Rushita Ferguson, Bradley Stratton, Matthew. The sequence listing filed with the application follows.

SEQUENCE LISTING (2 sequences)

SEQ ID NO: 1 - protein, 800 aa, Homo sapiens
MLQNVTPHNKLPGEGNAGLLGLGPEAAAPGKRIRKPSLLYEGFESPTMASVPALQLTPANPPPPEVSNPKKPGRVTNQLQYLHKVVMKALWKHQFAWPFRQPVDAVKLGLPDYHKIIKQPMDMGTIKRRLENNYYWAASECMQDFNTMFTNCYIYNKPTDDIVLMAQTLEKIFLQKVASMPQEEQELVVTIPKNSHKKGAKLAALQGSVTSAHQVPAVSSVSHTALYTPPPEIPTTVLNIPHPSVISSPLLKSLHSAGPPLLAVTAAPPAQPLAKKKGVKRKADTTTPTPTAILAPGSPASPPGSLEPKAARLPPMRRESGRPIKPPRKDLPDSQQQHQSSKKGKLSEQLKHCNGILKELLSKKHAAYAWPFYKPVDASALGLHDYHDIIKHPMDLSTVKRKMENRDYRDAQEFAADVRLMFSNCYKYNPPDHDVVAMARKLQDVFEFRYAKMPDEPLEPGPLPVSTAMPPGLAKSSSESSSEESSSESSSEEEEEEDEEDEEEEESESSDSEEERAHRLAELQEQLRAVHEQLAALSQGPISKPKRKREKKEKKKKRKAEKHRGRAGADEDDKGPRAPRPPQPKKSKKASGSGGGSAALGPSGFGPSGGSGTKLPKKATKTAPPALPTGYDSEEEEESRPMSYDEKRQLSLDINKLPGEKLGRVVHIIQAREPSLRDSNPEEIEIDFETLKPSTLRELERYVLSCLRKKPRKPYTIKKPVGKTKEELALEKKRELEKRLQDVSGQLNSTKKPPKKANEKTESSSAQQVAVSRLSASSSSSDSSSSSSSSSSSDTSDSDS

SEQ ID NO: 2 - protein, 347 aa, Homo sapiens
MLHTTQLYQHVPETRWPIVYSPRYNITFMGLEKLHPFDAGKWGKVINFLKEEKLLSDSMLVEAREASEEDLLVVHTRRYLNELKWSFAVATITEIPPVIFLPNFLVQRKVLRPLRTQTGGTIMAGKLAVERGWAINVGGGFHHCSSDRGGGFCAYADITLAIKFLFERVEGISRATIIDLDAHQGNGHERDFMDDKRVYIMDVYNRHIYPGDRFAKQAIRRKVELEWGTEDDEYLDKVERNIKKSLQEHLPDVVVYNAGTDILEGDRLGGLSISPAGIVKRDELVFRMVRGRRVPILMVTSGGYQKRTARIIADSILNLFGLGLIGPESPSVSAQNSDTPLLPPAVP